European Patent Specification EP 3 504 342 B1, published May 20, 2026. Title: NUCLEIC ACID EXTRACTION AND AMPLIFICATION CONTROLS AND METHODS OF USE THEREOF. Applicant: LIFE TECHNOLOGIES CORPORATION PAGANI, Ioanna ZERINGER, Emily LI, Kelly HUANG, Boli. Application Unassigned. The sequence listing filed with the application follows.

SEQUENCE LISTING (34 sequences)

SEQ ID NO: 1 - DNA, 18 bp, Artificial Sequence
  Synthetic DNA
gagcgtgtaactgttaaa

SEQ ID NO: 2 - DNA, 18 bp, Artificial Sequence
  Synthetic DNA
tttgcataatgaatctga

SEQ ID NO: 3 - DNA, 18 bp, Artificial Sequence
  Synthetic DNA
aagtgtgatgtttaaatc

SEQ ID NO: 4 - DNA, 18 bp, Artificial Sequence
  Synthetic DNA
gacaagaatgcctctgtc

SEQ ID NO: 5 - DNA, 18 bp, Artificial Sequence
  Synthetic DNA
gcctgttgaaatcgcaat

SEQ ID NO: 6 - DNA, 18 bp, Artificial Sequence
  Synthetic DNA
agcgattgaaatttatcc

SEQ ID NO: 7 - DNA, 18 bp, Artificial Sequence
  Synthetic DNA
ggtgaccttcatcgtgct

SEQ ID NO: 8 - DNA, 18 bp, Artificial Sequence
  Synthetic DNA
taggctatcaattaaatg

SEQ ID NO: 9 - DNA, 18 bp, Artificial Sequence
  Synthetic DNA
agttgctatcggttatcg

SEQ ID NO: 10 - DNA, 18 bp, Artificial Sequence
  Synthetic DNA
agttgctatcggttatcg

SEQ ID NO: 11 - DNA, 18 bp, Artificial Sequence
  Synthetic DNA
aggttttttatcatcctt

SEQ ID NO: 12 - DNA, 18 bp, Artificial Sequence
  Synthetic DNA
gttatatgttatttgttg

SEQ ID NO: 13 - DNA, 18 bp, Artificial Sequence
  Synthetic DNA
ggcgtaaagggcgcgcag

SEQ ID NO: 14 - DNA, 18 bp, Artificial Sequence
  Synthetic DNA
acgggacgaacggcaagg

SEQ ID NO: 15 - DNA, 18 bp, Artificial Sequence
  Synthetic DNA
acatctgttccaaaatct

SEQ ID NO: 16 - DNA, 18 bp, Artificial Sequence
  Synthetic DNA
acttgttggggatactta

SEQ ID NO: 17 - DNA, 18 bp, Artificial Sequence
  Synthetic DNA
acttccattccaaatctt

SEQ ID NO: 18 - DNA, 18 bp, Artificial Sequence
  Synthetic DNA
tgaattctttgttagaaa

SEQ ID NO: 19 - DNA, 18 bp, Artificial Sequence
  Synthetic DNA
gaagtaaaactgtattac

SEQ ID NO: 20 - DNA, 18 bp, Artificial Sequence
  Synthetic DNA
ggcaacggtggcttagtg

SEQ ID NO: 21 - DNA, 18 bp, Artificial Sequence
  Synthetic DNA
gtataaacgagacacact

SEQ ID NO: 22 - DNA, 18 bp, Artificial Sequence
  Synthetic DNA
gaaacagatacgacgtgg

SEQ ID NO: 23 - DNA, 18 bp, Artificial Sequence
  Synthetic DNA
gtgaactccgtattgaag

SEQ ID NO: 24 - DNA, 18 bp, Artificial Sequence
  Synthetic DNA
tttgatgatcctgacata

SEQ ID NO: 25 - DNA, 18 bp, Artificial Sequence
  Synthetic DNA
gtggagttttaactcatt

SEQ ID NO: 26 - DNA, 18 bp, Artificial Sequence
  Synthetic DNA
aaactgatggcgattatg

SEQ ID NO: 27 - DNA, 18 bp, Artificial Sequence
  Synthetic DNA
ccaccacaacttcagatt

SEQ ID NO: 28 - DNA, 18 bp, Artificial Sequence
  Synthetic DNA
ttcagggacgcttggcgg

SEQ ID NO: 29 - DNA, 18 bp, Artificial Sequence
  Synthetic DNA
gtcgaactgatggtggcc

SEQ ID NO: 30 - DNA, 18 bp, Artificial Sequence
  Synthetic DNA
agatggaacaccaacact

SEQ ID NO: 31 - DNA, 18 bp, Artificial Sequence
  Synthetic DNA
gtgatacatggtaagaaa

SEQ ID NO: 32 - DNA, 18 bp, Artificial Sequence
  Synthetic DNA
gctgctgaatcagtcgaa

SEQ ID NO: 33 - DNA, 18 bp, Artificial Sequence
  Synthetic DNA
acaggaggtcagtgtctg

SEQ ID NO: 34 - DNA, 18 bp, Artificial Sequence
  Synthetic DNA
cgggatagcgtcttgttg